European Patent Application EP 4 190 338 A1, published June 7, 2023. Title: Stem cell-derived exosome-containing composition and method for manufacturing the same. Applicant: Brexogen Inc. The sequence listing filed with the application follows.

SEQUENCE LISTING (24 sequences)

SEQ ID NO: 1 - DNA, 24 bp, Artificial Sequence
  TNF-a_primer1
gagctgaacaataggctgttccca

SEQ ID NO: 2 - DNA, 24 bp, Artificial Sequence
  TNF-a_primer2
agaggctcagcaatgagtgacagt

SEQ ID NO: 3 - DNA, 21 bp, Artificial Sequence
  IL-1b_primer1
acagctggagagtgtagatcc

SEQ ID NO: 4 - DNA, 21 bp, Artificial Sequence
  IL-1b_primer2
cttgagaggtgctgatgtacc

SEQ ID NO: 5 - DNA, 20 bp, Artificial Sequence
  IL-6_primer1
acagccactcacctcttcag

SEQ ID NO: 6 - DNA, 21 bp, Artificial Sequence
  IL-6_primer2
ccatctttttcagccatcttt

SEQ ID NO: 7 - DNA, 20 bp, Artificial Sequence
  CD206_primer1
cacgatccgacccttccttg

SEQ ID NO: 8 - DNA, 20 bp, Artificial Sequence
  CD206_primer2
gcttgcagtatgtctccgct

SEQ ID NO: 9 - DNA, 19 bp, Artificial Sequence
  ARG-1_primer1
cggagaccacagtttggca

SEQ ID NO: 10 - DNA, 20 bp, Artificial Sequence
  ARG-1_primer2
cctggcacatcgggaatctt

SEQ ID NO: 11 - DNA, 20 bp, Artificial Sequence
  IL-10_primer1
tgaaaacaagagcaaggccg

SEQ ID NO: 12 - DNA, 20 bp, Artificial Sequence
  IL-10_primer2
gccaccctgatgtctcagtt

SEQ ID NO: 13 - DNA, 22 bp, Artificial Sequence
  a-SMA _primer1
cccagacatcagggagtaatgg

SEQ ID NO: 14 - DNA, 22 bp, Artificial Sequence
  a-SMA _primer2
tctatcggatacttcagcgtca

SEQ ID NO: 15 - DNA, 19 bp, Artificial Sequence
  CTGF_primer1
cttctgcgatttcggctcc

SEQ ID NO: 16 - DNA, 19 bp, Artificial Sequence
  CTGF_primer2
tacaccgacccaccgaaga

SEQ ID NO: 17 - DNA, 20 bp, Artificial Sequence
  cTNT_primer1
agtgggaagaggcagactga

SEQ ID NO: 18 - DNA, 20 bp, Artificial Sequence
  cTNT_primer2
cgaacttctctgcctccaag

SEQ ID NO: 19 - DNA, 20 bp, Artificial Sequence
  hERG_primer1
caacctgggcgaccagatag

SEQ ID NO: 20 - DNA, 20 bp, Artificial Sequence
  hERG_primer2
ggtgttgggagagacgttgc

SEQ ID NO: 21 - DNA, 22 bp, Artificial Sequence
  Nav1.7_primer1
ggtttcagcacagattcaggtc

SEQ ID NO: 22 - DNA, 22 bp, Artificial Sequence
  Nav1.7_primer2
ccagctgaaagtgtcaaagctc

SEQ ID NO: 23 - DNA, 22 bp, Artificial Sequence
  MYH7_primer1
ctttgctgttattgcagccatt

SEQ ID NO: 24 - DNA, 21 bp, Artificial Sequence
  MYH7_primer2
agatgccaactttcctgttgc